European Patent Application EP 4 148 064 A1, published March 15, 2023. Title: Polypeptide Derivative Having Dual Receptor Agonistic Action and Use Thereof. Applicant: Tianjin Institute of Pharmaceutical Research Co., Ltd. Application EP21803512.9. The sequence listing filed with the application follows.

SEQUENCE LISTING (31 sequences)

SEQ ID NO: 1 - protein, 30 aa, Homo sapiens
  GLP-1
HAEGTFTSDVSSYLEGQAAKEFIAWLVKGR

SEQ ID NO: 2 - protein, 29 aa, Homo sapiens
  Glucagon
HSQGTFTSDYSKYLDSRRAQDFVQWLMNT

SEQ ID NO: 3 - protein, 37 aa, Homo sapiens
  Oxyntomodulin
HSQGTFTSDYSKYLDSRRAQDFVQWLMNTKRNRNNIA

SEQ ID NO: 4 - protein, 30 aa, Artificial Sequence
  Glucagon-derived peptide
  BINDING 20..20: The side chain of Lys is modified
HSQGTFTSDYSKYLDERAAKEFIAWLEAGG

SEQ ID NO: 5 - protein, 30 aa, Artificial Sequence
  Glucagon-derived peptide
  MUTAGEN 2..2: Serine is D-Ser
  BINDING 20..20: The side chain of Lys is modified
HSQGTFTSDYSKYLEEKAAKEFIAWLEAGG

SEQ ID NO: 6 - protein, 30 aa, Artificial Sequence
  Glucagon-derived peptide
  MUTAGEN 2..2: Serine is D-Ser
  BINDING 20..20: The side chain of Lys is modified
HSQGTFTSDYSKYLEERAAKEFIAWLEAGG

SEQ ID NO: 7 - protein, 30 aa, Artificial Sequence
  Glucagon-derived peptide
  MUTAGEN 2..2: Xaa is alpha-aminoisobutyric acid
  BINDING 20..20: The side chain of Lys is modified
HXQGTFTSDYSKYLDERAAKEFIAWLEAGG

SEQ ID NO: 8 - protein, 30 aa, Artificial Sequence
  Glucagon-derived peptide
  MUTAGEN 2..2: Xaa is alpha-aminoisobutyric acid
  BINDING 20..20: The side chain of Lys is modified
HXQGTFTSDYSKYLEERAAKEFIAWLEAGG

SEQ ID NO: 9 - protein, 30 aa, Artificial Sequence
  Glucagon-derived peptide
  MUTAGEN 2..2: Xaa is alpha-aminoisobutyric acid
  BINDING 20..20: The side chain of Lys is modified
HXQGTFTSDYSKYLDERAAKEFVAWLEAGG

SEQ ID NO: 10 - protein, 30 aa, Artificial Sequence
  Glucagon-derived peptide
  BINDING 20..20: The side chain of Lys is modified
HSQGTFTSDYSKYLDERAAKEFIAWLESGG

SEQ ID NO: 11 - protein, 30 aa, Artificial Sequence
  Glucagon-derived peptide
  MUTAGEN 2..2: Serine is D-Ser
  BINDING 20..20: The side chain of Lys is modified
HSQGTFTSDYSKYLEERAAKEFVAWLESGG

SEQ ID NO: 12 - protein, 30 aa, Artificial Sequence
  Glucagon-derived peptide
  MUTAGEN 2..2: Xaa is alpha-aminoisobutyric acid
  BINDING 20..20: The side chain of Lys is modified
HXQGTFTSDYSKYLDERAAKEFIAWLESGG

SEQ ID NO: 13 - protein, 30 aa, Artificial Sequence
  Glucagon-derived peptide
  MUTAGEN 2..2: Xaa is alpha-aminoisobutyric acid
  BINDING 20..20: The side chain of Lys is modified
HXQGTFTSDYSKYLEERAAKEFIAWLESGG

SEQ ID NO: 14 - protein, 30 aa, Artificial Sequence
  Glucagon-derived peptide
  MUTAGEN 2..2: Xaa is alpha-aminoisobutyric acid
  BINDING 20..20: The side chain of Lys is modified
HXQGTFTSDYSKYLEEKAAKEFVAWLESGG

SEQ ID NO: 15 - protein, 30 aa, Artificial Sequence
  Glucagon-derived peptide
  MUTAGEN 2..2: Xaa is alpha-aminoisobutyric acid
  BINDING 20..20: The side chain of Lys is modified
HXQGTFTSDYSKYLDEKAAKEFIAWLESGG

SEQ ID NO: 16 - protein, 29 aa, Artificial Sequence
  Glucagon-derived peptide
  BINDING 20..20: The side chain of Lys is modified
HSQGTFTSDYSKYLDERAAKEFIAWLEGG

SEQ ID NO: 17 - protein, 29 aa, Artificial Sequence
  Glucagon-derived peptide
  MUTAGEN 2..2: Serine is D-Ser
  BINDING 20..20: The side chain of Lys is modified
HSQGTFTSDYSKYLEERAAKEFVAWLEGG

SEQ ID NO: 18 - protein, 29 aa, Artificial Sequence
  Glucagon-derived peptide
  MUTAGEN 2..2: Xaa is alpha-aminoisobutyric acid
  BINDING 20..20: The side chain of Lys is modified
HXQGTFTSDYSKYLDERAAKEFIAWLEGG

SEQ ID NO: 19 - protein, 29 aa, Artificial Sequence
  Glucagon-derived peptide
  MUTAGEN 2..2: Xaa is alpha-aminoisobutyric acid
  BINDING 20..20: The side chain of Lys is modified
HXQGTFTSDYSKYLEERAAKEFIAWLEGG

SEQ ID NO: 20 - protein, 29 aa, Artificial Sequence
  Glucagon-derived peptide
  MUTAGEN 2..2: Xaa is alpha-aminoisobutyric acid
  BINDING 20..20: The side chain of Lys is modified
HXQGTFTSDYSKYLEEKAAKEFVAWLEGG

SEQ ID NO: 21 - protein, 29 aa, Artificial Sequence
  Glucagon-derived peptide
  MUTAGEN 2..2: Xaa is alpha-aminoisobutyric acid
  BINDING 20..20: The side chain of Lys is modified
HXQGTFTSDYSKYLDEKAAKEFIAWLEGG

SEQ ID NO: 22 - protein, 30 aa, Artificial Sequence
  Glucagon-derived peptide
  BINDING 20..20: The side chain of Lys is modified
HSQGTFTSDYSKYLDERAAKEFIAWLEGEG

SEQ ID NO: 23 - protein, 30 aa, Artificial Sequence
  Glucagon-derived peptide
  MUTAGEN 2..2: Serine is D-Ser
  BINDING 20..20: The side chain of Lys is modified
HSQGTFTSDYSKYLEEKAAKEFVAWLEGEG

SEQ ID NO: 24 - protein, 30 aa, Artificial Sequence
  Glucagon-derived peptide
  MUTAGEN 2..2: Xaa is alpha-aminoisobutyric acid
  BINDING 20..20: The side chain of Lys is modified
HXQGTFTSDYSKYLDERAAKEFIAWLEGEG

SEQ ID NO: 25 - protein, 30 aa, Artificial Sequence
  Glucagon-derived peptide
  MUTAGEN 2..2: Xaa is alpha-aminoisobutyric acid
  BINDING 20..20: The side chain of Lys is modified
HXQGTFTSDYSKYLEERAAKEFIAWLEGEG

SEQ ID NO: 26 - protein, 30 aa, Artificial Sequence
  Glucagon-derived peptide
  MUTAGEN 2..2: Xaa is alpha-aminoisobutyric acid
  BINDING 20..20: The side chain of Lys is modified
HXQGTFTSDYSKYLEEKAAKEFVAWLEGEG

SEQ ID NO: 27 - protein, 30 aa, Artificial Sequence
  Glucagon-derived peptide
  MUTAGEN 2..2: Xaa is alpha-aminoisobutyric acid
  BINDING 20..20: The side chain of Lys is modified
HXQGTFTSDYSKYLDEKAAKEFIAWLEGEG

SEQ ID NO: 28 - protein, 31 aa, Homo sapiens
  GLP-1
HAEGTFTSDVSSYLEGQAAKEFIAWLVKGRG

SEQ ID NO: 29 - protein, 10 aa, Artificial Sequence
  C terminus 10 peptides of Exendin-4
GPSSGAPPPS

SEQ ID NO: 30 - protein, 8 aa, Homo sapiens
  C-terminal inserted peptide fragment of OXM sequence
KRNRNNIA

SEQ ID NO: 31 - protein, 6 aa, Artificial Sequence
  Peptide fragment
GGPSSG